European Patent Application EP 4 163 289 A1, published April 12, 2023. Title: Peptide compound targeting elastin-derived peptides and  use thereof. Applicant: Shenzhen Turier Biotech. Co.,Ltd. The sequence listing filed with the application follows.

SEQUENCE LISTING (26 sequences)

SEQ ID NO: 1 - protein, 14 aa, Artificial
VVGSPSAQDEASPL

SEQ ID NO: 2 - protein, 14 aa, Artificial
VVGSPSAQDEASPA

SEQ ID NO: 3 - protein, 14 aa, Artificial
  MISC_FEATURE (2)..(2): Xaa=Iva
VXGSPSAQDEASPL

SEQ ID NO: 4 - protein, 14 aa, Artificial
VVGSPSAQEEASPL

SEQ ID NO: 5 - protein, 14 aa, Artificial
  MISC_FEATURE (2)..(2): Xaa=Iva
VXGSPSAQDEASPA

SEQ ID NO: 6 - protein, 14 aa, Artificial
  MISC_FEATURE (2)..(2): Xaa=Iva
VXGSPSAQDEASPA

SEQ ID NO: 7 - protein, 14 aa, Artificial
  MISC_FEATURE (2)..(2): Xaa=Iva
VXGSPSAQEEASPA

SEQ ID NO: 8 - protein, 14 aa, Artificial
  MISC_FEATURE (2)..(2): Xaa=Iva
VXGSPSAQEEASPA

SEQ ID NO: 9 - protein, 14 aa, Artificial
  MISC_FEATURE (2)..(2): Xaa=Iva
VXGSPSAQEDASPA

SEQ ID NO: 10 - protein, 15 aa, Artificial
EVVGSPSAQEDASPA

SEQ ID NO: 11 - protein, 14 aa, Artificial
  MISC_FEATURE (2)..(2): Xaa=Iva
VXGSPSAQEEASPL

SEQ ID NO: 12 - protein, 14 aa, Artificial
VVGSPSAQEDASPL

SEQ ID NO: 13 - protein, 14 aa, Artificial
  MISC_FEATURE (2)..(2): Xaa=Iva
VXGSPSAQEEASPA

SEQ ID NO: 14 - protein, 14 aa, Artificial
  MISC_FEATURE (2)..(2): Xaa=Iva
VXGSPSAQEEASPA

SEQ ID NO: 15 - protein, 14 aa, Artificial
  MISC_FEATURE (2)..(2): Xaa=Iva
VXGSPSAQEEASPA

SEQ ID NO: 16 - protein, 14 aa, Artificial
  MISC_FEATURE (2)..(2): Xaa=Iva
VXGSPSAQDEASPA

SEQ ID NO: 17 - protein, 14 aa, Artificial
VVGSPSAQDEASPL

SEQ ID NO: 18 - protein, 14 aa, Artificial
VVGSPSAQDEASPA

SEQ ID NO: 19 - protein, 14 aa, Artificial
  MISC_FEATURE (2)..(2): Xaa=Iva
  MISC_FEATURE (2)..(2): Xaa=Iva
VXGSPSAQDEASPL

SEQ ID NO: 20 - protein, 14 aa, Artificial
VVGSPSAQEEASPL

SEQ ID NO: 21 - protein, 14 aa, Artificial
  MISC_FEATURE (2)..(2): Xaa=Iva
VXGSPSAQDEASPA

SEQ ID NO: 22 - protein, 14 aa, Artificial
  MISC_FEATURE (2)..(2): Xaa=Iva
VXGSPSAQEEASPA

SEQ ID NO: 23 - protein, 14 aa, Artificial
  MISC_FEATURE (2)..(2): Xaa=Iva
VXGSPSAQEDASPL

SEQ ID NO: 24 - protein, 14 aa, Artificial
VVGSPSAQEDASPA

SEQ ID NO: 25 - protein, 14 aa, Artificial
  MISC_FEATURE (2)..(2): Xaa=Iva
VXGSPSAQEDASPA

SEQ ID NO: 26 - protein, 14 aa, Artificial
  MISC_FEATURE (2)..(2): Xaa=Val or Iva
  MISC_FEATURE (9)..(9): Xaa=Asp or Glu
  MISC_FEATURE (10)..(10): Xaa=Glu or Asp
  MISC_FEATURE (14)..(14): Xaa=Leu or Ala
VXGSPSAQXXASPX